European Patent Application EP 4 349 979 A1, published April 10, 2024. Title: ENGINEERED CAS12I NUCLEASE, EFFECTOR PROTEIN AND USE THEREOF. Applicant: INSTITUTE OF ZOOLOGY, CHINESE ACADEMY OF SCIENCES BEIJING INSTITUTE FOR STEM CELL AND REGENERATIVE MEDICINE. The sequence listing filed with the application follows.

SEQUENCE LISTING (79 sequences)

SEQ ID NO: 1 - protein, 1054 aa, Artificial Sequence
  synthetic sequence
MSSAIKSYKSVLRPNERKNQLLKSTIQCLEDGSAFFFKMLQGLFGGITPEIVRFSTEQEKQQQDIALWCAVNWFRPVSQDSLTHTIASDNLVEKFEEYYGGTASDAIKQYFSASIGESYYWNDCRQQYYDLCRELGVEVSDLTHDLEILCREKCLAVATESNQNNSIISVLFGTGEKEDRSVKLRITKKILEAISNLKEIPKNVAPIQEIILNVAKATKETFRQVYAGNLGAPSTLEKFIAKDGQKEFDLKKLQTDLKKVIRGKSKERDWCCQEELRSYVEQNTIQYDLWAWGEMFNKAHTALKIKSTRNYNFAKQRLEQFKEIQSLNNLLVVKKLNDFFDSEFFSGEETYTICVHHLGGKDLSKLYKAWEDDPADPENAIVVLCDDLKNNFKKEPIRNILRYIFTIRQECSAQDILAAAKYNQQLDRYKSQKANPSVLGNQGFTWTNAVILPEKAQRNDRPNSLDLRIWLYLKLRHPDGRWKKHHIPFYDTRFFQEIYAAGNSPVDTCQFRTPRFGYHLPKLTDQTAIRVNKKHVKAAKTEARIRLAIQQGTLPVSNLKITEISATINSKGQVRIPVKFDVGRQKGTLQIGDRFCGYDQNQTASHAYSLWEVVKEGQYHKELGCFVRFISSGDIVSITENRGNQFDQLSYEGLAYPQYADWRKKASKFVSLWQITKKNKKKEIVTVEAKEKFDAICKYQPRLYKFNKEYAYLLRDIVRGKSLVELQQIRQEIFRFIEQDCGVTRLGSLSLSTLETVKAVKGIIYSYFSTALNASKNNPISDEQRKEFDPELFALLEKLELIRTRKKKQKVERIANSLIQTCLENNIKFIRGEGDLSTTNNATKKKANSRSMDWLARGVFNKIRQLAPMHNITLFGCGSLYTSHQDPLVHRNPDKAMKCRWAAIPVKDIGDWVLRKLSQNLRAKNIGTGEYYHQGVKEFLSHYELQDLEEELLKWRSDRKSNIPCWVLQNRLAEKLGNKEAVVYIPVRGGRIYFATHKVATGAVSIVFDQKQVWVCNADHVAAANIALTVKGIGEQSSDEENPDGSRIKLQLTS

SEQ ID NO: 2 - protein, 1054 aa, Artificial Sequence
  synthetic sequence
MSSAIKSYKSVLRPNERKNQLLKSTIQCLEDGSAFFFKMLQGLFGGITPEIVRFSTEQEKQQQDIALWCAVNWFRPVSQDSLTHTIASDNLVEKFEEYYGGTASDAIKQYFSASIGESYYWNDCRQQYYDLCRELGVEVSDLTHDLEILCREKCLAVATESNQYNSIISVLFGTGRKEDRSVKLRITKKILEAISNLKEIPKNVAPIQEIILNVAKATKETFRQVYAGNLGAPSTLERFIAKDGQKEFDLKKLQTDLKKVIRGKSKERDWCCQEELRSYVEQNTIQYDLWAWGEMFNKAHTALKIKSTRNYNFAKQRLEQFKEIQSLNNLLVVKKLNDFFDSEFFSGEETYTICVHHLGGKDLSKLYKAWEDDPADPENAIVVLCDDLKNNFKKEPIRNILRYIFTIRQECSAQDILAAAKYNQQLDRYKSQKANPSVLGNQGFTWRNAVILPEKAQRNDRPNSLDLRIWLYLKLRHPDGRWKKHHIPFYDTRFFQEIYAAGNSPVDTCQFRTPRFGYHLPKLTDQTAIRVNKKHVKAAKTEARIRLAIQQGTLPVSNLKITRISATINSKGQVRIPVKFDVGRQKGTLQIGDRFCGYDQNQTASHAYSLWEVVKEGQYHKELGCFVRFISSGDIVSITENRGNQFDQLSYEGLAYPQYADWRKKASKFVSLWQITKKNKKKEIVTVEAKEKFDAICKYQPRLYKFNKEYAYLLRDIVRGKSLVELQQIRQEIFRFIEQDCGVTRLGSLSLSTLETVKAVKGIIYSYFSTALNASKNNPISDEQRKEFDPELFALLEKLELIRTRKKKQKVERIANSLIQTCLENNIKFIRGEGDLSTTNNATKKKANSRSMDWLARGVFNKIRQLAPMHNITLFGCGSLYTSHQDPLVHRNPDKAMKCRWAAIPVKDIGDWVLRKLSQNLRAKNIGTGEYYHQGVKEFLSHYELQDLEEELLKWRSDRKSNIPCWVLQNRLAEKLGNKEAVVYIPVRGGRIYFATHKVATGAVSIVFDQKQVWVCNADHVAAANIALTVKGIGEQSSDEENPDGSRIKLQLTS

SEQ ID NO: 3 - protein, 1054 aa, Artificial Sequence
  synthetic sequence
MSSAIKSYKSVLRPNERKNQLLKSTIQCLEDGSAFFFKMLQGLFGGITPEIVRFSTEQEKQQQDIALWCAVNWFRPVSQDSLTHTIASDNLVEKFEEYYGGTASDAIKQYFSASIGESYYWNDCRQQYYDLCRELGVEVSDLTHDLEILCREKCLAVATESNQNNSIISVLFGTGRKEDRSVKLRITKKILEAISNLKEIPKNVAPIQEIILNVAKATKETFRQVYAGNLGAPSTLERFIAKDGQKEFDLKKLQTDLKKVIRGKSKERDWCCQEELRSYVEQNTIQYDLWAWGEMFNKAHTALKIKSTRNYNFAKQRLEQFKEIQSLNNLLVVKKLNDFFDSEFFSGEETYTICVHHLGGKDLSKLYKAWEDDPADPENAIVVLCDDLKNNFKKEPIRNILRYIFTIRQECSAQDILAAAKYNQQLDRYKSQKANPSVLGNQGFTWRNAVILPEKAQRNDRPNSLDLRIWLYLKLRHPDGRWKKHHIPFYDTRFFQEIYAAGNSPVDTCQFRTPRFGYHLPKLTDQTAIRVNKKHVKAAKTEARIRLAIQQGTLPVSNLKITRISATINSKGQVRIPVKFDVGRQKGTLQIGDRFCGYDQNQTASHAYSLWEVVKEGQYHKELGCFVRFISSGDIVSITENRGNQFDQLSYEGLAYPQYADWRKKASKFVSLWQITKKNKKKEIVTVEAKEKFDAICKYQPRLYKFNKEYAYLLRDIVRGKSLVELQQIRQEIFRFIEQDCGVTRLGSLSLSTLETVKAVKGIIYSYFSTALNASKNNPISDEQRKEFDPELFALLEKLELIRTRKKKQKVERIANSLIQTCLENNIKFIRGEGDLSTTNNATKKKANSRSMDWLARGVFNKIRQLAPMHNITLFGCGSLYTSHQDPLVHRNPDKAMKCRWAAIPVKDIGDWVLRKLSQNLRAKNRGTGEYYHQGVKEFLSHYELQDLEEELLKWRSDRKSNIPCWVLQNRLAEKLGNKEAVVYIPVRGGRIYFATHKVATGAVSIVFDQKQVWVCNADHVAAANIALTVKGIGEQSSDEENPDGSRIKLQLTS

SEQ ID NO: 4 - protein, 1054 aa, Artificial Sequence
  synthetic sequence
MSSAIKSYKSVLRPNERKNQLLKSTIQCLEDGSAFFFKMLQGLFGGITPEIVRFSTEQEKQQQDIALWCAVNWFRPVSQDSLTHTIASDNLVEKFEEYYGGTASDAIKQYFSASIGESYYWNDCRQQYYDLCRELGVEVSDLTHDLEILCREKCLAVATESNQNNSIISVLFGTGRKEDRSVKLRITKKILEAISNLKEIPKNVAPIQEIILNVAKATKETFRQVYAGNLGAPSTLERFIAKDGQKEFDLKKLQTDLKKVIRGKSKERDWCCQEELRSYVEQNTIQYDLWAWGEMFNKAHTALKIKSTRNYNFAKQRLEQFKRIQSLNNLLVVKKLNDFFDSEFFSGEETYTICVHHLGGKRLSKLYKAWEDDPADPENAIVVLCDDLKNNFKKEPIRNILRYIFTIRQECSAQDILAAAKYNQQLDRYKSQKANPSVLGNQGFTWRNAVILPEKAQRNDRPNSLDLRIWLYLKLRHPDGRWKKHHIPFYDTRFFQEIYAAGNSPVDTCQFRTPRFGYHLPKLTDQTAIRVNKKHVKAAKTEARIRLAIQQGTLPVSNLKITRISATINSKGQVRIPVKFDVGRQKGTLQIGDRFCGYDQNQTASHAYSLWEVVKEGQYHKELGCFVRFISSGDIVSITENRGNQFDQLSYEGLAYPQYADWRKKASKFVSLWQITKKNKKKEIVTVEAKEKFDAICKYQPRLYKFNKEYAYLLRDIVRGKSLVELQQIRQEIFRFIEQDCGVTRLGSLSLSTLETVKAVKGIIYSYFSTALNASKNNPISDEQRKEFDPELFALLEKLELIRTRKKKQKVERIANSLIQTCLENNIKFIRGEGDLSTTNNATKKKANSRSMDWLARGVFNKIRQLAPMHNITLFGCGSLYTSHQDPLVHRNPDKAMKCRWAAIPVKDIGDWVLRKLSQNLRAKNIGTGEYYHQGVKEFLSHYELQDLEEELLKWRSDRKSNIPCWVLQNRLAEKLGNKEAVVYIPVRGGRIYFATHKVATGAVSIVFDQKQVWVCNADHVAAANIALTVKGIGEQSSDEENPDGSRIKLQLTS

SEQ ID NO: 5 - protein, 1054 aa, Artificial Sequence
  synthetic sequence
MSSAIKSYKSVLRPNERKNQLLKSTIQCLEDGSAFFFKMLQGLFGGITPEIVRFSTEQEKQQQDIALWCAVNWFRPVSQDSLTHTIASDNLVEKFEEYYGGTASDAIKQYFSASIGESYYWNDCRQQYYDLCRELGVEVSDLTHDLEILCREKCLAVATESNQYNSIISVLFGTGEKEDRSVKLRITKKILEAISNLKEIPKNVAPIQEIILNVAKATKETFRQVYAGNLGAPSTLEKFIAKDGQKEFDLKKLQTDLKKVIRGKSKERDWCCQEELRSYVEQNTIQYDLWAWGEMFNKAHTALKIKSTRNYNFAKQRLEQFKEIQSLNNLLVVKKLNDFFDSEFFSGEETYTICVHHLGGKDLSKLYKAWEDDPADPENAIVVLCDDLKNNFKKEPIRNILRYIFTIRQECSAQDILAAAKYNQQLDRYKSQKANPSVLGNQGFTWTNAVILPEKAQRNDRPNSLDLRIWLYLKLRHPDGRWKKHHIPFYDTRFFQEIYAAGNSPVDTCQFRTPRFGYHLPKLTDQTAIRVNKKHVKAAKTEARIRLAIQQGTLPVSNLKITEISATINSKGQVRIPVKFDVGRQKGTLQIGDRFCGYDQNQTASHAYSLWEVVKEGQYHKELGCFVRFISSGDIVSITENRGNQFDQLSYEGLAYPQYADWRKKASKFVSLWQITKKNKKKEIVTVEAKEKFDAICKYQPRLYKFNKEYAYLLRDIVRGKSLVELQQIRQEIFRFIEQDCGVTRLGSLSLSTLETVKAVKGIIYSYFSTALNASKNNPISDEQRKEFDPELFALLEKLELIRTRKKKQKVERIANSLIQTCLENNIKFIRGEGDLSTTNNATKKKANSRSMDWLARGVFNKIRQLAPMHNITLFGCGSLYTSHQDPLVHRNPDKAMKCRWAAIPVKDIGDWVLRKLSQNLRAKNRGTGEYYHQGVKEFLSHYELQDLEEELLKWRSDRKSNIPCWVLQNRLAEKLGNKEAVVYIPVRGGRIYFATHKVATGAVSIVFDQKQVWVCNADHVAAANIALTVKGIGEQSSDEENPDGSRIKLQLTS

SEQ ID NO: 6 - protein, 1054 aa, Artificial Sequence
  synthetic sequence
MSSAIKSYKSVLRPNERKNQLLKSTIQCLEDGSAFFFKMLQGLFGGITPEIVRFSTEQEKQQQDIALWCAVNWFRPVSQDSLTHTIASDNLVEKFEEYYGGTASDAIKQYFSASIGESYYWNDCRQQYYDLCRELGVEVSDLTHDLEILCREKCLAVATESNQYNSIISVLFGTGEKEDRSVKLRITKKILEAISNLKEIPKNVAPIQEIILNVAKATKETFRQVYAGNLGAPSTLEKFIAKDGQKEFDLKKLQTDLKKVIRGKSKERDWCCQEELRSYVEQNTIQYDLWAWGEMFNKAHTALKIKSTRNYNFAKQRLEQFKRIQSLNNLLVVKKLNDFFDSEFFSGEETYTICVHHLGGKRLSKLYKAWEDDPADPENAIVVLCDDLKNNFKKEPIRNILRYIFTIRQECSAQDILAAAKYNQQLDRYKSQKANPSVLGNQGFTWTNAVILPEKAQRNDRPNSLDLRIWLYLKLRHPDGRWKKHHIPFYDTRFFQEIYAAGNSPVDTCQFRTPRFGYHLPKLTDQTAIRVNKKHVKAAKTEARIRLAIQQGTLPVSNLKITEISATINSKGQVRIPVKFDVGRQKGTLQIGDRFCGYDQNQTASHAYSLWEVVKEGQYHKELGCFVRFISSGDIVSITENRGNQFDQLSYEGLAYPQYADWRKKASKFVSLWQITKKNKKKEIVTVEAKEKFDAICKYQPRLYKFNKEYAYLLRDIVRGKSLVELQQIRQEIFRFIEQDCGVTRLGSLSLSTLETVKAVKGIIYSYFSTALNASKNNPISDEQRKEFDPELFALLEKLELIRTRKKKQKVERIANSLIQTCLENNIKFIRGEGDLSTTNNATKKKANSRSMDWLARGVFNKIRQLAPMHNITLFGCGSLYTSHQDPLVHRNPDKAMKCRWAAIPVKDIGDWVLRKLSQNLRAKNIGTGEYYHQGVKEFLSHYELQDLEEELLKWRSDRKSNIPCWVLQNRLAEKLGNKEAVVYIPVRGGRIYFATHKVATGAVSIVFDQKQVWVCNADHVAAANIALTVKGIGEQSSDEENPDGSRIKLQLTS

SEQ ID NO: 7 - protein, 1054 aa, Artificial Sequence
  synthetic sequence
MSSAIKSYKSVLRPNERKNQLLKSTIQCLEDGSAFFFKMLQGLFGGITPEIVRFSTEQEKQQQDIALWCAVNWFRPVSQDSLTHTIASDNLVEKFEEYYGGTASDAIKQYFSASIGESYYWNDCRQQYYDLCRELGVEVSDLTHDLEILCREKCLAVATESNQYNSIISVLFGTGRKEDRSVKLRITKKILEAISNLKEIPKNVAPIQEIILNVAKATKETFRQVYAGNLGAPSTLERFIAKDGQKEFDLKKLQTDLKKVIRGKSKERDWCCQEELRSYVEQNTIQYDLWAWGEMFNKAHTALKIKSTRNYNFAKQRLEQFKEIQSLNNLLVVKKLNDFFDSEFFSGEETYTICVHHLGGKDLSKLYKAWEDDPADPENAIVVLCDDLKNNFKKEPIRNILRYIFTIRQECSAQDILAAAKYNQQLDRYKSQKANPSVLGNQGFTWRNAVILPEKAQRNDRPNSLDLRIWLYLKLRHPDGRWKKHHIPFYDTRFFQEIYAAGNSPVDTCQFRTPRFGYHLPKLTDQTAIRVNKKHVKAAKTEARIRLAIQQGTLPVSNLKITRISATINSKGQVRIPVKFDVGRQKGTLQIGDRFCGYDQNQTASHAYSLWEVVKEGQYHKELGCFVRFISSGDIVSITENRGNQFDQLSYEGLAYPQYADWRKKASKFVSLWQITKKNKKKEIVTVEAKEKFDAICKYQPRLYKFNKEYAYLLRDIVRGKSLVELQQIRQEIFRFIEQDCGVTRLGSLSLSTLETVKAVKGIIYSYFSTALNASKNNPISDEQRKEFDPELFALLEKLELIRTRKKKQKVERIANSLIQTCLENNIKFIRGEGDLSTTNNATKKKANSRSMDWLARGVFNKIRQLAPMHNITLFGCGSLYTSHQDPLVHRNPDKAMKCRWAAIPVKDIGDWVLRKLSQNLRAKNRGTGEYYHQGVKEFLSHYELQDLEEELLKWRSDRKSNIPCWVLQNRLAEKLGNKEAVVYIPVRGGRIYFATHKVATGAVSIVFDQKQVWVCNADHVAAANIALTVKGIGEQSSDEENPDGSRIKLQLTS

SEQ ID NO: 8 - protein, 1054 aa, Artificial Sequence
  synthetic sequence
MSSAIKSYKSVLRPNERKNQLLKSTIQCLEDGSAFFFKMLQGLFGGITPEIVRFSTEQEKQQQDIALWCAVNWFRPVSQDSLTHTIASDNLVEKFEEYYGGTASDAIKQYFSASIGESYYWNDCRQQYYDLCRELGVEVSDLTHDLEILCREKCLAVATESNQYNSIISVLFGTGRKEDRSVKLRITKKILEAISNLKEIPKNVAPIQEIILNVAKATKETFRQVYAGNLGAPSTLERFIAKDGQKEFDLKKLQTDLKKVIRGKSKERDWCCQEELRSYVEQNTIQYDLWAWGEMFNKAHTALKIKSTRNYNFAKQRLEQFKRIQSLNNLLVVKKLNDFFDSEFFSGEETYTICVHHLGGKRLSKLYKAWEDDPADPENAIVVLCDDLKNNFKKEPIRNILRYIFTIRQECSAQDILAAAKYNQQLDRYKSQKANPSVLGNQGFTWRNAVILPEKAQRNDRPNSLDLRIWLYLKLRHPDGRWKKHHIPFYDTRFFQEIYAAGNSPVDTCQFRTPRFGYHLPKLTDQTAIRVNKKHVKAAKTEARIRLAIQQGTLPVSNLKITRISATINSKGQVRIPVKFDVGRQKGTLQIGDRFCGYDQNQTASHAYSLWEVVKEGQYHKELGCFVRFISSGDIVSITENRGNQFDQLSYEGLAYPQYADWRKKASKFVSLWQITKKNKKKEIVTVEAKEKFDAICKYQPRLYKFNKEYAYLLRDIVRGKSLVELQQIRQEIFRFIEQDCGVTRLGSLSLSTLETVKAVKGIIYSYFSTALNASKNNPISDEQRKEFDPELFALLEKLELIRTRKKKQKVERIANSLIQTCLENNIKFIRGEGDLSTTNNATKKKANSRSMDWLARGVFNKIRQLAPMHNITLFGCGSLYTSHQDPLVHRNPDKAMKCRWAAIPVKDIGDWVLRKLSQNLRAKNIGTGEYYHQGVKEFLSHYELQDLEEELLKWRSDRKSNIPCWVLQNRLAEKLGNKEAVVYIPVRGGRIYFATHKVATGAVSIVFDQKQVWVCNADHVAAANIALTVKGIGEQSSDEENPDGSRIKLQLTS

SEQ ID NO: 9 - protein, 1054 aa, Artificial Sequence
  synthetic sequence
MSSAIKSYKSVLRPNERKNQLLKSTIQCLEDGSAFFFKMLQGLFGGITPEIVRFSTEQEKQQQDIALWCAVNWFRPVSQDSLTHTIASDNLVEKFEEYYGGTASDAIKQYFSASIGESYYWNDCRQQYYDLCRELGVEVSDLTHDLEILCREKCLAVATESNQYNSIISVLFGTGRKEDRSVKLRITKKILEAISNLKEIPKNVAPIQEIILNVAKATKETFRQVYAGNLGAPSTLERFIAKDGQKEFDLKKLQTDLKKVIRGKSKERDWCCQEELRSYVEQNTIQYDLWAWGEMFNKAHTALKIKSTRNYNFAKQRLEQFKRIQSLNNLLVVKKLNDFFDSEFFSGEETYTICVHHLGGKRLSKLYKAWEDDPADPENAIVVLCDDLKNNFKKEPIRNILRYIFTIRQECSAQDILAAAKYNQQLDRYKSQKANPSVLGNQGFTWRNAVILPEKAQRNDRPNSLDLRIWLYLKLRHPDGRWKKHHIPFYDTRFFQEIYAAGNSPVDTCQFRTPRFGYHLPKLTDQTAIRVNKKHVKAAKTEARIRLAIQQGTLPVSNLKITRISATINSKGQVRIPVKFDVGRQKGTLQIGDRFCGYDQNQTASHAYSLWEVVKEGQYHKELGCFVRFISSGDIVSITENRGNQFDQLSYEGLAYPQYADWRKKASKFVSLWQITKKNKKKEIVTVEAKEKFDAICKYQPRLYKFNKEYAYLLRDIVRGKSLVELQQIRQEIFRFIEQDCGVTRLGSLSLSTLETVKAVKGIIYSYFSTALNASKNNPISDEQRKEFDPELFALLEKLELIRTRKKKQKVERIANSLIQTCLENNIKFIRGEGDLSTTNNATKKKANSRSMDWLARGVFNKIRQLAPMHNITLFGCGSLYTSHQDPLVHRNPDKAMKCRWAAIPVKDIGDWVLRKLSQNLRAKNRGTGEYYHQGVKEFLSHYELQDLEEELLKWRSDRKSNIPCWVLQNRLAEKLGNKEAVVYIPVRGGRIYFATHKVATGAVSIVFDQKQVWVCNADHVAAANIALTVKGIGEQSSDEENPDGSRIKLQLTS

SEQ ID NO: 10 - protein, 1054 aa, Artificial Sequence
  synthetic sequence
MSSAIKSYKSVLRPNERKNQLLKSTIQCLEDGSAFFFKMLQGLFGGITPEIVRFSTEQEKQQQDIALWCAVNWFRPVSQDSLTHTIASDNLVEKFEEYYGGTASDAIKQYFSASIGESYYWNDCRQQYYDLCRELGVEVSDLTHDLEILCREKCLAVATESNQYNSIISVLFGTGRKEDRSVKLRITKKILEAISNLKEIPKNVAPIQEIILNVAKATKETFRQVYAGNLGAPSTLERFIAKDGQKEFDLKKLQTDLKKVIRGKSKERDWCCQEELRSYVEQNTIQYDLWAWGEMFNKAHTALKIKSTRNYNFAKQRLEQFKRIQSLNNLLVVKKLNDFFDSEFFSGEETYTICVHHLGGKRLSKLYKAWEDDPADPENAIVVLCDDLKNNFKKEPIRNILRYIFTIRQECSAQDILAAAKYNQQLDRYKSQKANPSVLGNQGFTWRNAVILPEKAQRNDRPNSLDLRIWLYLKLRHPDGRWKKHHIPFYDTRFFQEIYAAGNSPVDTCQFRTPRFGYHLPKLTDQTAIRVNKKHVKAAKTEARIRLAIQQGTLPVSNLKITRISATINSKGQVRIPVKFDVGRQKGTLQIGDRFCGYDQNQTASHAYSLWEVVKEGQYHKELGCFVRFISSGDIVSITENRGNQFDQLSYEGLAYPQYADWRKKASKFVSLWQITKKNKKKEIVTVEAKEKFDAICKYQPRLYKFNKEYAYLLRDIVRGKSLVELQQIRQEIFRFIEQDCGVTRLGSLSLSTLETVKAVKGIIYSYFSTALNASKNNPISDEQRKEFDPELFALLEKLELIRTRKKKQKVERIANSLIQTCLENNIKFIRGEGDLSTTNNATKKKANSRSMDWLARGVFNKIRQLAPMHNITLFGCGSLYTSHQDPLVHRNPDKAMKCRWAAIPVKDIGDWVLRKLSQNLRAKNGGTGEYYHQGVKEFLSHYELQDLEEELLKWRSDRKSNIPCWVLQNRLAEKLGNKEAVVYIPVRGGRIYFATHKVATGAVSIVFDQKQVWVCNADHVAAANIALTVKGIGEQSSDEENPDGSRIKLQLTS

SEQ ID NO: 11 - protein, 1056 aa, Artificial Sequence
  synthetic sequence
MSSAIKSYKSVLRPNERKNQLLKSTIQCLEDGSAFFFKMLQGLFGGITPEIVRFSTEQEKQQQDIALWCAVNWFRPVSQDSLTHTIASDNLVEKFEEYYGGTASDAIKQYFSASIGESYYWNDCRQQYYDLCRELGVEVSDLTHDLEILCREKCLAVATESNQYNSIISVLFGTGRKEDRSVKLRITKKILEAISNLKEIPKNVAPIQEIILNVAKATKETFRQVYAGNLGAPSTLERFIAKDGQKEFDLKKLQTDLKKVIRGKSKERDWCCQEELRSYVEQNTIQYDLWAWGEMFNKAHTALKIKSTRNYNFAKQRLEQFKRIQSLNNLLVVKKLNDFFDSEFFSGEETYTICVHHLGGKRLSKLYKAWEDDPADPENAIVVLCDDLKNNFKKEPIRNILRYIFTIRQECSAQDILAAAKYNQQLDRYKSQKANPSVLGGGNQGFTWRNAVILPEKAQRNDRPNSLDLRIWLYLKLRHPDGRWKKHHIPFYDTRFFQEIYAAGNSPVDTCQFRTPRFGYHLPKLTDQTAIRVNKKHVKAAKTEARIRLAIQQGTLPVSNLKITRISATINSKGQVRIPVKFDVGRQKGTLQIGDRFCGYDQNQTASHAYSLWEVVKEGQYHKELGCFVRFISSGDIVSITENRGNQFDQLSYEGLAYPQYADWRKKASKFVSLWQITKKNKKKEIVTVEAKEKFDAICKYQPRLYKFNKEYAYLLRDIVRGKSLVELQQIRQEIFRFIEQDCGVTRLGSLSLSTLETVKAVKGIIYSYFSTALNASKNNPISDEQRKEFDPELFALLEKLELIRTRKKKQKVERIANSLIQTCLENNIKFIRGEGDLSTTNNATKKKANSRSMDWLARGVFNKIRQLAPMHNITLFGCGSLYTSHQDPLVHRNPDKAMKCRWAAIPVKDIGDWVLRKLSQNLRAKNGGTGEYYHQGVKEFLSHYELQDLEEELLKWRSDRKSNIPCWVLQNRLAEKLGNKEAVVYIPVRGGRIYFATHKVATGAVSIVFDQKQVWVCNADHVAAANIALTVKGIGEQSSDEENPDGSRIKLQLTS

SEQ ID NO: 12 - protein, 1055 aa, Artificial Sequence
  synthetic sequence
MSSAIKSYKSVLRPNERKNQLLKSTIQCLEDGSAFFFKMLQGLFGGITPEIVRFSTEQEKQQQDIALWCAVNWFRPVSQDSLTHTIASDNLVEKFEEYYGGTASDAIKQYFSASIGESYYWNDCRQQYYDLCRELGVEVSDLTHDLEILCREKCLAVATESNQYNSIISVLFGTGRKEDRSVKLRITKKILEAISNLKEIPKNVAPIQEIILNVAKATKETFRQVYAGNLGAPSTLERFIAKDGQKEFDLKKLQTDLKKVIRGKSKERDWCCQEELRSYVEQNTIQYDLWAWGEMFNKAHTALKIKSTRNYNFAKQRLEQFKRIQSLNNLLVVKKLNDFFDSEFFSGEETYTICVHHLGGKRLSKLYKAWEDDPADPENAIVVLCDDLKNNFKKEPIRNILRYIFTIRQECSAQDILAAAKYNQQLDRYKSQKANPSVLGGNQGFTWRNAVILPEKAQRNDRPNSLDLRIWLYLKLRHPDGRWKKHHIPFYDTRFFQEIYAAGNSPVDTCQFRTPRFGYHLPKLTDQTAIRVNKKHVKAAKTEARIRLAIQQGTLPVSNLKITRISATINSKGQVRIPVKFDVGRQKGTLQIGDRFCGYDQNQTASHAYSLWEVVKEGQYHKELGCFVRFISSGDIVSITENRGNQFDQLSYEGLAYPQYADWRKKASKFVSLWQITKKNKKKEIVTVEAKEKFDAICKYQPRLYKFNKEYAYLLRDIVRGKSLVELQQIRQEIFRFIEQDCGVTRLGSLSLSTLETVKAVKGIIYSYFSTALNASKNNPISDEQRKEFDPELFALLEKLELIRTRKKKQKVERIANSLIQTCLENNIKFIRGEGDLSTTNNATKKKANSRSMDWLARGVFNKIRQLAPMHNITLFGCGSLYTSHQDPLVHRNPDKAMKCRWAAIPVKDIGDWVLRKLSQNLRAKNGGTGEYYHQGVKEFLSHYELQDLEEELLKWRSDRKSNIPCWVLQNRLAEKLGNKEAVVYIPVRGGRIYFATHKVATGAVSIVFDQKQVWVCNADHVAAANIALTVKGIGEQSSDEENPDGSRIKLQLTS

SEQ ID NO: 13 - protein, 1093 aa, Artificial Sequence
  synthetic sequence
MSNKEKNASETRKAYTTKMIPRSHDRMKLLGNFMDYLMDGTPIFFELWNQFGGGIDRDIISGTANKDKISDDLLLAVNWFKVMPINSKPQGVSPSNLANLFQQYSGSEPDIQAQEYFASNFDTEKHQWKDMRVEYERLLAELQLSRSDMHHDLKLMYKEKCIGLSLSTAHYITSVMFGTGAKNNRQTKHQFYSKVIQLLEESTQINSVEQLASIILKAGDCDSYRKLRIRCSRKGATPSILKIVQDYELGTNHDDEVNVPSLIANLKEKLGRFEYECEWKCMEKIKAFLASKVGPYYLGSYSAMLENALSPIKGMTTKNCKFVLKQIDAKNDIKYENEPFGKIVEGFFDSPYFESDTNVKWVLHPHHIGESNIKTLWEDLNAIHSKYEEDIASLSEDKKEKRIKVYQGDVCQTINTYCEEVGKEAKTPLVQLLRYLYSRKDDIAVDKIIDGITFLSKKHKVEKQKINPVIQKYPSFNFGNNSKLLGKIISPKDKLKHNLKCNRNQVDNYIWIEIKVLNTKTMRWEKHHYALSSTRFLEEVYYPATSENPPDALAARFRTKTNGYEGKPALSAEQIEQIRSAPVGLRKVKKRQMRLEAARQQNLLPRYTWGKDFNINICKRGNNFEVTLATKVKKKKEKNYKVVLGYDANIVRKNTYAAIEAHANGDGVIDYNDLPVKPIESGFVTVESQVRDKSYDQLSYNGVKLLYCKPHVESRRSFLEKYRNGTMKDNRGNNIQIDFMKDFEAIADDETSLYYFNMKYCKLLQSSIRNHSSQAKEYREEIFELLRDGKLSVLKLSSLSNLSFVMFKVAKSLIGTYFGHLLKKPKNSKSDVKAPPITDEDKQKADPEMFALRLALEEKRLNKVKSKKEVIANKIVAKALELRDKYGPVLIKGENISDTTKKGKKSSTNSFLMDWLARGVANKVKEMVMMHQGLEFVEVNPNFTSHQDPFVHKNPENTFRARYSRCTPSELTEKNRKEILSFLSDKPSKRPTNAYYNEGAMAFLATYGLKKNDVLGVSLEKFKQIMANILHQRSEDQLLFPSRGGMFYLATYKLDADATSVNWNGKQFWVCNADLVAAYNVGLVDIQKDFKKK

SEQ ID NO: 14 - protein, 1054 aa, Artificial Sequence
  synthetic sequence
MSSAIKSYKSVLRPNERKNQLLKSTIQCLEDGSAFFFKMLQGLFGGITPEIVRFSTEQEKQQQDIALWCAVNWFRPVSQDSLTHTIASDNLVEKFEEYYGGTASDAIKQYFSASIGESYYWNDCRQQYYDLCRELGVEVSDLTHDLEILCREKCLAVATESNQYNSIISVLFGTGRKEDRSVKLRITKKILEAISNLKEIPKNVAPIQEIILNVAKATKETFRQVYAGNLGAPSTLERFIAKDGQKEFDLKKLQTDLKKVIRGKSKERDWCCQEELRSYVEQNTIQYDLWAWGEMFNKAHTALKIKSTRNYNFAKQRLEQFKRIQSLNNLLVVKKLNDFFDSEFFSGEETYTICVHHLGGKRLSKLYKAWEDDPADPENAIVVLCDDLKNNFKKEPIRNILRYIFTIRQECSAQDILAAAKYNQQLDRYKSQKANPSVLGNQGFTWRNAVILPEKAQRNDRPNSLDLRIWLYLKLRHPDGRWKKHHIPFYDTRFFQEIYAAGNSPVDTCQFRTPRFGYHLPKLTDQTAIRVNKKHVKAAKTEARIRLAIQQGTLPVSNLKITRISATINSKGQVRIPVKFDVGRQKGTLQIGDRFCGYDQNQTASHAYSLWEVVKEGQYHKELGCFVRFISSGDIVSITENRGNQFDQLSYEGLAYPQYADWRKKASKFVSLWQITKKNKKKEIVTVEAKEKFDAICKYQPRLYKFNKEYAYLLRDIVRGKSLVELQQIRQEIFRFIEQDCGVTRLGSLSLSTLETVKAVKGIIYSYFSTALNASKNNPISDEQRKEFDPELFALLEKLELIRTRKKKQKVERIANSLIQTCLENNIKFIRGEGDLSTTNNATKKKANSRSMDWLAAGVFNKIRQLAPMHNITLFGCGSLYTSHQDPLVHRNPDKAMKCRWAAIPVKDIGDWVLRKLSQNLRAKNIGTGEYYHQGVKEFLSHYELQDLEEELLKWRSDRKSNIPCWVLQNRLAEKLGNKEAVVYIPVRGGRIYFATHKVATGAVSIVFDQKQVWVCNADHVAAANIALTVKGIGEQSSDEENPDGSRIKLQLTS

SEQ ID NO: 15 - protein, 1054 aa, Artificial Sequence
  synthetic sequence
MSSAIKSYKSVLRPNERKNQLLKSTIQCLEDGSAFFFKMLQGLFGGITPEIVRFSTEQEKQQQDIALWCAVNWFRPVSQDSLTHTIASDNLVEKFEEYYGGTASDAIKQYFSASIGESYYWNDCRQQYYDLCRELGVEVSDLTHDLEILCREKCLAVATESNQYNSIISVLFGTGRKEDRSVKLRITKKILEAISNLKEIPKNVAPIQEIILNVAKATKETFRQVYAGNLGAPSTLERFIAKDGQKEFDLKKLQTDLKKVIRGKSKERDWCCQEELRSYVEQNTIQYDLWAWGEMFNKAHTALKIKSTRNYNFAKQRLEQFKRIQSLNNLLVVKKLNDFFDSEFFSGEETYTICVHHLGGKRLSKLYKAWEDDPADPENAIVVLCDDLKNNFKKEPIRNILRYIFTIRQECSAQDILAAAKYNQQLDRYKSQKANPSVLGNQGFTWRNAVILPEKAQRNDRPNSLDLRIWLYLKLRHPDGRWKKHHIPFYDTRFFQEIYAAGNSPVDTCQFRTPRFGYHLPKLTDQTAIRVNKKHVKAAKTEARIRLAIQQGTLPVSNLKITRISATINSKGQVRIPVKFDVGRQKGTLQIGDRFCGYDQNQTASHAYSLWEVVKEGQYHKELGCFVRFISSGDIVSITENRGNQFDQLSYEGLAYPQYADWRKKASKFVSLWQITKKNKKKEIVTVEAKEKFDAICKYQPRLYKFNKEYAYLLRDIVRGKSLVELQQIRQEIFRFIEQDCGVTRLGSLSLSTLETVKAVKGIIYSYFSTALNASKNNPISDEQRKEFDPELFALLEKLELIRTRKKKQKVERIANSLIQTCLENNIKFIRGEGDLSTTNNATKKKANSRSMDWLARGVFAKIRQLAPMHNITLFGCGSLYTSHQDPLVHRNPDKAMKCRWAAIPVKDIGDWVLRKLSQNLRAKNIGTGEYYHQGVKEFLSHYELQDLEEELLKWRSDRKSNIPCWVLQNRLAEKLGNKEAVVYIPVRGGRIYFATHKVATGAVSIVFDQKQVWVCNADHVAAANIALTVKGIGEQSSDEENPDGSRIKLQLTS

SEQ ID NO: 16 - protein, 1054 aa, Artificial Sequence
  synthetic sequence
MSSAIKSYKSVLRPNERKNQLLKSTIQCLEDGSAFFFKMLQGLFGGITPEIVRFSTEQEKQQQDIALWCAVNWFRPVSQDSLTHTIASDNLVEKFEEYYGGTASDAIKQYFSASIGESYYWNDCRQQYYDLCRELGVEVSDLTHDLEILCREKCLAVATESNQYNSIISVLFGTGRKEDRSVKLRITKKILEAISNLKEIPKNVAPIQEIILNVAKATKETFRQVYAGNLGAPSTLERFIAKDGQKEFDLKKLQTDLKKVIRGKSKERDWCCQEELRSYVEQNTIQYDLWAWGEMFNKAHTALKIKSTRNYNFAKQRLEQFKRIQSLNNLLVVKKLNDFFDSEFFSGEETYTICVHHLGGKRLSKLYKAWEDDPADPENAIVVLCDDLKNNFKKEPIRNILRYIFTIRQECSAQDILAAAKYNQQLDRYKSQKANPSVLGNQGFTWRNAVILPEKAQRNDRPNSLDLRIWLYLKLRHPDGRWKKHHIPFYDTRFFQEIYAAGNSPVDTCQFRTPRFGYHLPKLTDQTAIRVNKKHVKAAKTEARIRLAIQQGTLPVSNLKITRISATINSKGQVRIPVKFDVGRQKGTLQIGDRFCGYDQNQTASHAYSLWEVVKEGQYHKELGCFVRFISSGDIVSITENRGNQFDQLSYEGLAYPQYADWRKKASKFVSLWQITKKNKKKEIVTVEAKEKFDAICKYQPRLYKFNKEYAYLLRDIVRGKSLVELQQIRQEIFRFIEQDCGVTRLGSLSLSTLETVKAVKGIIYSYFSTALNASKNNPISDEQRKEFDPELFALLEKLELIRTRKAKQKVERIANSLIQTCLENNIKFIRGEGDLSTTNNATKKKANSRSMDWLARGVFNKIRQLAPMHNITLFGCGSLYTSHQDPLVHRNPDKAMKCRWAAIPVKDIGDWVLRKLSQNLRAKNIGTGEYYHQGVKEFLSHYELQDLEEELLKWRSDRKSNIPCWVLQNRLAEKLGNKEAVVYIPVRGGRIYFATHKVATGAVSIVFDQKQVWVCNADHVAAANIALTVKGIGEQSSDEENPDGSRIKLQLTS

SEQ ID NO: 17 - protein, 1054 aa, Artificial Sequence
  synthetic sequence
MSSAIKSYKSVLRPNERKNQLLKSTIQCLEDGSAFFFKMLQGLFGGITPEIVRFSTEQEKQQQDIALWCAVNWFRPVSQDSLTHTIASDNLVEKFEEYYGGTASDAIKQYFSASIGESYYWNDCRQQYYDLCRELGVEVSDLTHDLEILCREKCLAVATESNQYNSIISVLFGTGRKEDRSVKLRITKKILEAISNLKEIPKNVAPIQEIILNVAKATKETFRQVYAGNLGAPSTLERFIAKDGQKEFDLKKLQTDLKKVIRGKSKERDWCCQEELRSYVEQNTIQYDLWAWGEMFNKAHTALKIKSTRNYNFAKQRLEQFKRIQSLNNLLVVKKLNDFFDSEFFSGEETYTICVHHLGGKRLSKLYKAWEDDPADPENAIVVLCDDLKNNFKKEPIRNILRYIFTIRQECSAQDILAAAKYNQQLDRYKSQKANPSVLGNQGFTWRNAVILPEKAQRNDRPNSLDLRIWLYLKLRHPDGRWKKHHIPFYDTRFFQEIYAAGNSPVDTCQFRTPRFGYHLPKLTDQTAIRVNKKHVKAAKTEARIRLAIQQGTLPVSNLKITRISATINSKGQVRIPVKFDVGRQKGTLQIGDRFCGYDQNQTASHAYSLWEVVKEGQYHKELGCFVRFISSGDIVSITENRGNQFDQLSYEGLAYPQYADWRKKASKFVSLWQITKKNKKKEIVTVEAKEKFDAICKYQPRLYKFNKEYAYLLRDIVRGKSLVELQQIRQEIFRFIEQDCGVTRLGSLSLSTLETVKAVKGIIYSYFSTALNASKNNPISDEQRKEFDPELFALLEKLELIRTRKKKQKVERIANSLIQTCLENNIKFIRGEGDLSTTNNATKKKAASRSMDWLARGVFNKIRQLAPMHNITLFGCGSLYTSHQDPLVHRNPDKAMKCRWAAIPVKDIGDWVLRKLSQNLRAKNIGTGEYYHQGVKEFLSHYELQDLEEELLKWRSDRKSNIPCWVLQNRLAEKLGNKEAVVYIPVRGGRIYFATHKVATGAVSIVFDQKQVWVCNADHVAAANIALTVKGIGEQSSDEENPDGSRIKLQLTS

SEQ ID NO: 18 - protein, 1054 aa, Artificial Sequence
  synthetic sequence
MSSAIKSYKSVLRPNERKNQLLKSTIQCLEDGSAFFFKMLQGLFGGITPEIVRFSTEQEKQQQDIALWCAVNWFRPVSQDSLTHTIASDNLVEKFEEYYGGTASDAIKQYFSASIGESYYWNDCRQQYYDLCRELGVEVSDLTHDLEILCREKCLAVATESNQYNSIISVLFGTGRKEDRSVKLRITKKILEAISNLKEIPKNVAPIQEIILNVAKATKETFRQVYAGNLGAPSTLERFIAKDGQKEFDLKKLQTDLKKVIRGKSKERDWCCQEELRSYVEQNTIQYDLWAWGEMFNKAHTALKIKSTRNYNFAKQRLEQFKRIQSLNNLLVVKKLNDFFDSEFFSGEETYTICVHHLGGKRLSKLYKAWEDDPADPENAIVVLCDDLKNNFKKEPIRNILRYIFTIRQECSAQDILAAAKYNQQLDRYKSQKANPSVLGNQGFTWRNAVILPEKAQRNDRPNSLDLRIWLYLKLRHPDGRWKKHHIPFYDTRFFQEIYAAGNSPVDTCQFRTPRFGYHLPKLTDQTAIRVNKKHVKAAKTEARIRLAIQQGTLPVSNLKITRISATINSKGQVRIPVKFDVGRQKGTLQIGDRFCGYDQNQTASHAYSLWEVVKEGQYHKELGCFVRFISSGDIVSITENRGNQFDQLSYEGLAYPQYADWRKKASKFVSLWQITKKNKKKEIVTVEAKEKFDAICKYQPRLYKFNKEYAYLLADIVRGKSLVELQQIRQEIFRFIEQDCGVTRLGSLSLSTLETVKAVKGIIYSYFSTALNASKNNPISDEQRKEFDPELFALLEKLELIRTRKKKQKVERIANSLIQTCLENNIKFIRGEGDLSTTNNATKKKANSRSMDWLARGVFNKIRQLAPMHNITLFGCGSLYTSHQDPLVHRNPDKAMKCRWAAIPVKDIGDWVLRKLSQNLRAKNIGTGEYYHQGVKEFLSHYELQDLEEELLKWRSDRKSNIPCWVLQNRLAEKLGNKEAVVYIPVRGGRIYFATHKVATGAVSIVFDQKQVWVCNADHVAAANIALTVKGIGEQSSDEENPDGSRIKLQLTS

SEQ ID NO: 19 - protein, 1054 aa, Artificial Sequence
  synthetic sequence
MSSAIKSYKSVLRPNERKNQLLKSTIQCLEDGSAFFFKMLQGLFGGITPEIVRFSTEQEKQQQDIALWCAVNWFRPVSQDSLTHTIASDNLVEKFEEYYGGTASDAIKQYFSASIGESYYWNDCRQQYYDLCRELGVEVSDLTHDLEILCREKCLAVATESNQYNSIISVLFGTGRKEDRSVKLRITKKILEAISNLKEIPKNVAPIQEIILNVAKATKETFRQVYAGNLGAPSTLERFIAKDGQKEFDLKKLQTDLKKVIRGKSKERDWCCQEELRSYVEQNTIQYDLWAWGEMFNKAHTALKIKSTRNYNFAKQRLEQFKRIQSLNNLLVVKKLNDFFDSEFFSGEETYTICVHHLGGKRLSKLYKAWEDDPADPENAIVVLCDDLKNNFKKEPIRNILRYIFTIRQECSAQDILAAAKYNQQLDRYKSQKANPSVLGNQGFTWRNAVILPEKAQRNDRPNSLDLRIWLYLKLRHPDGRWKKHHIPFYDTRFFQEIYAAGNSPVDTCQFRTPRFGYHLPKLTDQTAIRVNKKHVKAAKTEARIRLAIQQGTLPVSNLKITRISATINSKGQVRIPVKFDVGRQKGTLQIGDRFCGYDQNQTASHAYSLWEVVKEGQYHKELGCFVRFISSGDIVSITENRGNQFDQLSYEGLAYPQYADWRKKASKFVSLWQITKKNKKKEIVTVEAKEKFDAICKYQPRLYKFNKEYAYLLRDIVAGKSLVELQQIRQEIFRFIEQDCGVTRLGSLSLSTLETVKAVKGIIYSYFSTALNASKNNPISDEQRKEFDPELFALLEKLELIRTRKKKQKVERIANSLIQTCLENNIKFIRGEGDLSTTNNATKKKANSRSMDWLARGVFNKIRQLAPMHNITLFGCGSLYTSHQDPLVHRNPDKAMKCRWAAIPVKDIGDWVLRKLSQNLRAKNIGTGEYYHQGVKEFLSHYELQDLEEELLKWRSDRKSNIPCWVLQNRLAEKLGNKEAVVYIPVRGGRIYFATHKVATGAVSIVFDQKQVWVCNADHVAAANIALTVKGIGEQSSDEENPDGSRIKLQLTS

SEQ ID NO: 20 - protein, 1054 aa, Artificial Sequence
  synthetic sequence
MSSAIKSYKSVLRPNERKNQLLKSTIQCLEDGSAFFFKMLQGLFGGITPEIVRFSTEQEKQQQDIALWCAVNWFRPVSQDSLTHTIASDNLVEKFEEYYGGTASDAIKQYFSASIGESYYWNDCRQQYYDLCRELGVEVSDLTHDLEILCREKCLAVATESNQYNSIISVLFGTGRKEDRSVKLRITKKILEAISNLKEIPKNVAPIQEIILNVAKATKETFRQVYAGNLGAPSTLERFIAKDGQKEFDLKKLQTDLKKVIRGKSKERDWCCQEELRSYVEQNTIQYDLWAWGEMFNKAHTALKIKSTRNYNFAKQRLEQFKRIQSLNNLLVVKKLNDFFDSEFFSGEETYTICVHHLGGKRLSKLYKAWEDDPADPENAIVVLCDDLKNNFKAEPIRNILRYIFTIRQECSAQDILAAAKYNQQLDRYKSQKANPSVLGNQGFTWRNAVILPEKAQRNDRPNSLDLRIWLYLKLRHPDGRWKKHHIPFYDTRFFQEIYAAGNSPVDTCQFRTPRFGYHLPKLTDQTAIRVNKKHVKAAKTEARIRLAIQQGTLPVSNLKITRISATINSKGQVRIPVKFDVGRQKGTLQIGDRFCGYDQNQTASHAYSLWEVVKEGQYHKELGCFVRFISSGDIVSITENRGNQFDQLSYEGLAYPQYADWRKKASKFVSLWQITKKNKKKEIVTVEAKEKFDAICKYQPRLYKFNKEYAYLLRDIVRGKSLVELQQIRQEIFRFIEQDCGVTRLGSLSLSTLETVKAVKGIIYSYFSTALNASKNNPISDEQRKEFDPELFALLEKLELIRTRKKKQKVERIANSLIQTCLENNIKFIRGEGDLSTTNNATKKKANSRSMDWLARGVFNKIRQLAPMHNITLFGCGSLYTSHQDPLVHRNPDKAMKCRWAAIPVKDIGDWVLRKLSQNLRAKNIGTGEYYHQGVKEFLSHYELQDLEEELLKWRSDRKSNIPCWVLQNRLAEKLGNKEAVVYIPVRGGRIYFATHKVATGAVSIVFDQKQVWVCNADHVAAANIALTVKGIGEQSSDEENPDGSRIKLQLTS

SEQ ID NO: 21 - protein, 1054 aa, Artificial Sequence
  synthetic sequence
MSSAIKSYKSVLRPNERKNQLLKSTIQCLEDGSAFFFKMLQGLFGGITPEIVRFSTEQEKQQQDIALWCAVNWFRPVSQDSLTHTIASDNLVEKFEEYYGGTASDAIKQYFSASIGESYYWNDCRQQYYDLCRELGVEVSDLTHDLEILCREKCLAVATESNQYNSIISVLFGTGRKEDRSVKLRITKKILEAISNLKEIPKNVAPIQEIILNVAKATKETFRQVYAGNLGAPSTLERFIAKDGQKEFDLKKLQTDLKKVIRGKSKERDWCCQEELRSYVEQNTIQYDLWAWGEMFNKAHTALKIKSTRNYNFAKQRLEQFKRIQSLNNLLVVKKLNDFFDSEFFSGEETYTICVHALGGKRLSKLYKAWEDDPADPENAIVVLCDDLKNNFKKEPIRNILRYIFTIRQECSAQDILAAAKYNQQLDRYKSQKANPSVLGNQGFTWRNAVILPEKAQRNDRPNSLDLRIWLYLKLRHPDGRWKKHHIPFYDTRFFQEIYAAGNSPVDTCQFRTPRFGYHLPKLTDQTAIRVNKKHVKAAKTEARIRLAIQQGTLPVSNLKITRISATINSKGQVRIPVKFDVGRQKGTLQIGDRFCGYDQNQTASHAYSLWEVVKEGQYHKELGCFVRFISSGDIVSITENRGNQFDQLSYEGLAYPQYADWRKKASKFVSLWQITKKNKKKEIVTVEAKEKFDAICKYQPRLYKFNKEYAYLLRDIVRGKSLVELQQIRQEIFRFIEQDCGVTRLGSLSLSTLETVKAVKGIIYSYFSTALNASKNNPISDEQRKEFDPELFALLEKLELIRTRKKKQKVERIANSLIQTCLENNIKFIRGEGDLSTTNNATKKKANSRSMDWLARGVFNKIRQLAPMHNITLFGCGSLYTSHQDPLVHRNPDKAMKCRWAAIPVKDIGDWVLRKLSQNLRAKNIGTGEYYHQGVKEFLSHYELQDLEEELLKWRSDRKSNIPCWVLQNRLAEKLGNKEAVVYIPVRGGRIYFATHKVATGAVSIVFDQKQVWVCNADHVAAANIALTVKGIGEQSSDEENPDGSRIKLQLTS

SEQ ID NO: 22 - protein, 1054 aa, Artificial Sequence
  synthetic sequence
MSSAIKSYKSVLRPNERKNQLLKSTIQCLEDGSAFFFKMLQGLFGGITPEIVRFSTEQEKQQQDIALWCAVNWFRPVSQDSLTHTIASDNLVEKFEEYYGGTASDAIKQYFSASIGESYYWNDCRQQYYDLCRELGVEVSDLTHDLEILCREKCLAVATESNQYNSIISVLFGTGRKEDRSVKLRITKKILEAISNLKEIPKNVAPIQEIILNVAKATKETFRQVYAGNLGAPSTLERFIAKDGQKEFDLKKLQTDLKKVIRGKSKERDWCCQEELRSYVEQNTIQYDLWAWGEMFNKAHTALKIKSTRNYNFAKQRLEQFKRIQSLNNLLVVKKLNDFFDSEFFSGEETYTICVHHLGGKRLSKLYKAWEDDPADPENAIVVLCDDLKNNFKKEPIRNILRYIFTIRQECSAQDILAAAKYNQQLDRYKSQKANPSVLGNQGFTWRNAVILPEKAQRNDRPNSLDLRIWLYLKLRHPDGRWKKHHIPFYDTRFFQEIYAAGNSPVDTCQFRTPRFGYHLPKLTDQTAIRVNKKHVKAAKTEARIRLAIQQGTLPVSNLKITRISATINSKGQVRIPVKFDVGRQKGTLQIGDRFCGYDQNQTASHAYSLWEVVKEGQYHKELGCFVRFISSGDIVSITENRGNQFDQLSYEGLAYPQYADWRKKASKFVSLWQITKKNKKKEIVTVEAKEKFDAICKYQPRLYKFNKEYAYLLRDIVRGKSLVELQQIRQEIFRFIEQDCGVTRLGSLSLSTLETVKAVKGIIYSYFSTALNASKNNPISDEQRKEFDPELFALLEKLELIRTRKKKQKVERIANSLIQTCLENNIKFIRGEGDLSTTNNATAKKANSRSMDWLARGVFNKIRQLAPMHNITLFGCGSLYTSHQDPLVHRNPDKAMKCRWAAIPVKDIGDWVLRKLSQNLRAKNIGTGEYYHQGVKEFLSHYELQDLEEELLKWRSDRKSNIPCWVLQNRLAEKLGNKEAVVYIPVRGGRIYFATHKVATGAVSIVFDQKQVWVCNADHVAAANIALTVKGIGEQSSDEENPDGSRIKLQLTS

SEQ ID NO: 23 - protein, 1054 aa, Artificial Sequence
  synthetic sequence
MSSAIKSYKSVLRPNERKNQLLKSTIQCLEDGSAFFFKMLQGLFGGITPEIVRFSTEQEKQQQDIALWCAVNWFRPVSQDSLTHTIASDNLVEKFEEYYGGTASDAIKQYFSASIGESYYWNDCRQQYYDLCRELGVEVSDLTHDLEILCREKCLAVATESNQYNSIISVLFGTGRKEDRSVKLRITKKILEAISNLKEIPKNVAPIQEIILNVAKATKETFRQVYAGNLGAPSTLERFIAKDGQKEFDLKKLQTDLKKVIRGKSKERDWCCQEELRSYVEQNTIQYDLWAWGEMFNKAHTALKIKSTRNYNFAKQRLEQFKRIQSLNNLLVVKKLNDFFDSEFFSGEETYTICVHHLGGKRLSKLYKAWEDDPADPENAIVVLCDDLKNNFKKEPIRNILRYIFTIRQECSAQDILAAAKYNQQLDRYKSQKANPSVLGNQGFTWRNAVILPEKAQRNDRPNSLDLRIWLYLKLRHPDGRWKKHHIPFYDTRFFQEIYAAGNSPVDTCQFRTPRFGYHLPKLTDQTAIRVNKKHVKAAKTEARIRLAIQQGTLPVSNLKITRISATINSKGQVRIPVKFDVGRQKGTLQIGDRFCGYDQNQTASHAYSLWEVVKEGQYHKELGCFVRFISSGDIVSITENRGNQFDQLSYEGLAYPQYADWRKKASKFVSLWQITKKNKKKEIVTVEAKEKFDAICKYQPRLYKFNKEYAYLLRDIVAGKSLVELQQIRQEIFRFIEQDCGVTRLGSLSLSTLETVKAVKGIIYSYFSTALNASKNNPISDEQRKEFDPELFALLEKLELIRTRKKKQKVERIANSLIQTCLENNIKFIRGEGDLSTTNNATAKKANSRSMDWLARGVFNKIRQLAPMHNITLFGCGSLYTSHQDPLVHRNPDKAMKCRWAAIPVKDIGDWVLRKLSQNLRAKNIGTGEYYHQGVKEFLSHYELQDLEEELLKWRSDRKSNIPCWVLQNRLAEKLGNKEAVVYIPVRGGRIYFATHKVATGAVSIVFDQKQVWVCNADHVAAANIALTVKGIGEQSSDEENPDGSRIKLQLTS

SEQ ID NO: 24 - protein, 1054 aa, Artificial Sequence
  synthetic sequence
MSSAIKSYKSVLRPNERKNQLLKSTIQCLEDGSAFFFKMLQGLFGGITPEIVRFSTEQEKQQQDIALWCAVNWFRPVSQDSLTHTIASDNLVEKFEEYYGGTASDAIKQYFSASIGESYYWNDCRQQYYDLCRELGVEVSDLTHDLEILCREKCLAVATESNQYNSIISVLFGTGRKEDRSVKLRITKKILEAISNLKEIPKNVAPIQEIILNVAKATKETFRQVYAGNLGAPSTLERFIAKDGQKEFDLKKLQTDLKKVIRGKSKERDWCCQEELRSYVEQNTIQYDLWAWGEMFNKAHTALKIKSTRNYNFAKQRLEQFKRIQSLNNLLVVKKLNDFFDSEFFSGEETYTICVHHLGGKRLSKLYKAWEDDPADPENAIVVLCDDLKNNFKKEPIRNILRYIFTIRQECSAQDILAAAKYNQQLDRYKSQKANPSVLGNQGFTWRNAVILPEKAQRNDRPNSLDLRIWLYLKLRHPDGRWKKHHIPFYDTRFFQEIYAAGNSPVDTCQFRTPRFGYHLPKLTDQTAIRVNKKHVKAAKTEARIRLAIQQGTLPVSNLKITRISATINSKGQVRIPVKFDVGRQKGTLQIGDRFCGYDQNQTASHAYSLWEVVKEGQYHKELGCFVRFISSGDIVSITENRGNQFDQLSYEGLAYPQYADWRKKASKFVSLWQITKKNKKKEIVTVEAKEKFDAICKYQPRLYKFNKEYAYLLRDIVRGKSLVELQQIRQEIFRFIEQDCGVTRLGSLSLSTLETVKAVKGIIYSYFSTALNASKNNPISDEQRKEFDPELFALLEKLELIRTRKKKQKVERIANSLIQTCLENNIKFIRGEGDLSTTNNATAKKANSRSMDWLAAGVFNKIRQLAPMHNITLFGCGSLYTSHQDPLVHRNPDKAMKCRWAAIPVKDIGDWVLRKLSQNLRAKNIGTGEYYHQGVKEFLSHYELQDLEEELLKWRSDRKSNIPCWVLQNRLAEKLGNKEAVVYIPVRGGRIYFATHKVATGAVSIVFDQKQVWVCNADHVAAANIALTVKGIGEQSSDEENPDGSRIKLQLTS

SEQ ID NO: 25 - DNA, 34 bp, Artificial Sequence
  synthetic sequence
gtttaattgagttgtcatatgttaataacggtat

SEQ ID NO: 26 - DNA, 34 bp, Artificial Sequence
  synthetic sequence
ataccgttattaacatatgacaactcaattaaac

SEQ ID NO: 27 - DNA, 20 bp, Artificial Sequence
  synthetic sequence
tggttgcccaccctagtcat

SEQ ID NO: 28 - DNA, 20 bp, Artificial Sequence
  synthetic sequence
tggttgcccaccctagtcat

SEQ ID NO: 29 - DNA, 20 bp, Artificial Sequence
  synthetic sequence
tgtttgcccaccctagtcct

SEQ ID NO: 30 - DNA, 20 bp, Artificial Sequence
  synthetic sequence
tgattgcccaccctactcct

SEQ ID NO: 31 - DNA, 20 bp, Artificial Sequence
  synthetic sequence
tggtcacccaccctagtctg

SEQ ID NO: 32 - DNA, 20 bp, Artificial Sequence
  synthetic sequence
tacaggaggcaataacagat

SEQ ID NO: 33 - DNA, 20 bp, Artificial Sequence
  synthetic sequence
gccaggaggcaataacagat

SEQ ID NO: 34 - DNA, 20 bp, Artificial Sequence
  synthetic sequence
tacattaggcaataacagat

SEQ ID NO: 35 - DNA, 20 bp, Artificial Sequence
  synthetic sequence
tacaggaggcaataacctat

SEQ ID NO: 36 - DNA, 20 bp, Artificial Sequence
  synthetic sequence
tacaggaggcaataacagcg

SEQ ID NO: 37 - DNA, 20 bp, Artificial Sequence
  synthetic sequence
accttgtagatgaactcgcc

SEQ ID NO: 38 - DNA, 20 bp, Artificial Sequence
  synthetic sequence
cacttgtagatgaactcgcc

SEQ ID NO: 39 - DNA, 20 bp, Artificial Sequence
  synthetic sequence
acctgttagatgaactcgcc

SEQ ID NO: 40 - DNA, 20 bp, Artificial Sequence
  synthetic sequence
accttgtagatgaactcgaa

SEQ ID NO: 41 - DNA, 19 bp, Artificial Sequence
  synthetic sequence
taatacgactcactatagg

SEQ ID NO: 42 - DNA, 67 bp, Artificial Sequence
  synthetic sequence
aaaaatttgtttggatatgttgaaccgtcaatgaaagacggatttctccctatagtgagtcgtatta

SEQ ID NO: 43 - DNA, 24 bp, Artificial Sequence
  synthetic sequence
cttcttcaacatatccaaacaaat

SEQ ID NO: 44 - DNA, 24 bp, Artificial Sequence
  synthetic sequence
ctacttcaacatatccaaacaaat

SEQ ID NO: 45 - DNA, 24 bp, Artificial Sequence
  synthetic sequence
ctccttcaacatatccaaacaaat

SEQ ID NO: 46 - DNA, 24 bp, Artificial Sequence
  synthetic sequence
ctgcttcaacatatccaaacaaat

SEQ ID NO: 47 - DNA, 24 bp, Artificial Sequence
  synthetic sequence
catcttcaacatatccaaacaaat

SEQ ID NO: 48 - DNA, 24 bp, Artificial Sequence
  synthetic sequence
caacttcaacatatccaaacaaat

SEQ ID NO: 49 - DNA, 24 bp, Artificial Sequence
  synthetic sequence
caccttcaacatatccaaacaaat

SEQ ID NO: 50 - DNA, 24 bp, Artificial Sequence
  synthetic sequence
cagcttcaacatatccaaacaaat

SEQ ID NO: 51 - DNA, 24 bp, Artificial Sequence
  synthetic sequence
cctcttcaacatatccaaacaaat

SEQ ID NO: 52 - DNA, 24 bp, Artificial Sequence
  synthetic sequence
ccacttcaacatatccaaacaaat

SEQ ID NO: 53 - DNA, 24 bp, Artificial Sequence
  synthetic sequence
ccccttcaacatatccaaacaaat

SEQ ID NO: 54 - DNA, 24 bp, Artificial Sequence
  synthetic sequence
ccgcttcaacatatccaaacaaat

SEQ ID NO: 55 - DNA, 24 bp, Artificial Sequence
  synthetic sequence
cgtcttcaacatatccaaacaaat

SEQ ID NO: 56 - DNA, 24 bp, Artificial Sequence
  synthetic sequence
cgacttcaacatatccaaacaaat

SEQ ID NO: 57 - DNA, 24 bp, Artificial Sequence
  synthetic sequence
cgccttcaacatatccaaacaaat

SEQ ID NO: 58 - DNA, 24 bp, Artificial Sequence
  synthetic sequence
cggcttcaacatatccaaacaaat

SEQ ID NO: 59 - DNA, 23 bp, Artificial Sequence
  synthetic sequence
agaaatccgtctttcattgacgg

SEQ ID NO: 60 - DNA, 20 bp, Artificial Sequence
  synthetic sequence
aggccaaagaattcctggaa

SEQ ID NO: 61 - DNA, 20 bp, Artificial Sequence
  synthetic sequence
ttcaacatatccaaacaaat

SEQ ID NO: 62 - DNA, 20 bp, Artificial Sequence
  synthetic sequence
tcctgaacaccttccaggaa

SEQ ID NO: 63 - DNA, 20 bp, Artificial Sequence
  synthetic sequence
gtgggagatgttgcaaggct

SEQ ID NO: 64 - DNA, 20 bp, Artificial Sequence
  synthetic sequence
atgtcacttaggataggaga

SEQ ID NO: 65 - DNA, 20 bp, Artificial Sequence
  synthetic sequence
ttgcctcctgtaaaagagtc

SEQ ID NO: 66 - protein, 9 aa, Artificial Sequence
  synthetic sequence
PKKKRKVPG

SEQ ID NO: 67 - protein, 9 aa, Artificial Sequence
  synthetic sequence
ASPKKKRKV

SEQ ID NO: 68 - DNA, 17 bp, Artificial Sequence
  synthetic sequence
  misc_feature (6)..(11): any base
  misc_feature (6)..(6): n is a, c, g, t or u
  misc_feature (7)..(7): n is a, c, g, t or u
  misc_feature (8)..(8): n is a, c, g, t or u
  misc_feature (9)..(9): n is a, c, g, t or u
  misc_feature (10)..(10): n is a, c, g, t or u
  misc_feature (11)..(11): n is a, c, g, t or u
ccgucnnnnnnugacgg

SEQ ID NO: 69 - DNA, 17 bp, Artificial Sequence
  synthetic sequence
  misc_feature (6)..(11): any base
  misc_feature (6)..(6): n is a, c, g, t or u
  misc_feature (7)..(7): n is a, c, g, t or u
  misc_feature (8)..(8): n is a, c, g, t or u
  misc_feature (9)..(9): n is a, c, g, t or u
  misc_feature (10)..(10): n is a, c, g, t or u
  misc_feature (11)..(11): n is a, c, g, t or u
gugccnnnnnnuggcac

SEQ ID NO: 70 - DNA, 16 bp, Artificial Sequence
  synthetic sequence
  misc_feature (6)..(10): any base
  misc_feature (6)..(6): n is a, c, g, t or u
  misc_feature (7)..(7): n is a, c, g, t or u
  misc_feature (8)..(8): n is a, c, g, t or u
  misc_feature (9)..(9): n is a, c, g, t or u
  misc_feature (10)..(10): n is a, c, g, t or u
  misc_feature (16)..(16): c,t,u
gugucnnnnnugacan

SEQ ID NO: 71 - DNA, 17 bp, Artificial Sequence
  synthetic sequence
  misc_feature (6)..(11): any base
  misc_feature (6)..(6): n is a, c, g, t or u
  misc_feature (7)..(7): n is a, c, g, t or u
  misc_feature (8)..(8): n is a, c, g, t or u
  misc_feature (9)..(9): n is a, c, g, t or u
  misc_feature (10)..(10): n is a, c, g, t or u
  misc_feature (11)..(11): n is a, c, g, t or u
  misc_feature (17)..(17): c,t,u
gugucnnnnnnugacan

SEQ ID NO: 72 - DNA, 14 bp, Artificial Sequence
  synthetic sequence
  misc_feature (3)..(3): c,t,u
  misc_feature (5)..(5): a,t,u
  misc_feature (6)..(6): a,c,g
  misc_feature (7)..(7): a,g
ucnunnnuugacgg

SEQ ID NO: 73 - DNA, 14 bp, Artificial Sequence
  synthetic sequence
  misc_feature (3)..(3): c,t,u
  misc_feature (4)..(4): a,t,u
  misc_feature (5)..(5): c,t,u
  misc_feature (7)..(7): a,g
ccnnncnuuggcac

SEQ ID NO: 74 - protein, 2 aa, Artificial Sequence
  synthetic sequence
GS

SEQ ID NO: 75 - protein, 4 aa, Artificial Sequence
  synthetic sequence
GGGS

SEQ ID NO: 76 - protein, 5 aa, Artificial Sequence
  synthetic sequence
GGGGS

SEQ ID NO: 77 - DNA, 23 bp, Artificial Sequence
  synthetic sequence
  misc_feature (3)..(3): n is a, c, g, t or u
ttntggttgcccaccctagtcat

SEQ ID NO: 78 - DNA, 23 bp, Artificial Sequence
  synthetic sequence
  misc_feature (3)..(3): n is a, c, g, t or u
ttnaaccactagcactagccttg

SEQ ID NO: 79 - DNA, 36 bp, Artificial Sequence
  synthetic sequence
gttgcaaaacccaagaaatccgtctttcattgacgg